European Patent Application EP 4 726 042 A2, published April 15, 2026. Title: Antisense oligomers targeting SETD5 for upregulation and use thereof. Applicant: Korea Advanced Institute of Science and Technology. The sequence listing filed with the application follows.

SEQUENCE LISTING (174 sequences)

SEQ ID NO: 1 - DNA, 21 bp, Homo sapiens
  source 1..21: mol_type = genomic DNA
gcttacagaaaggaagtggaa

SEQ ID NO: 2 - DNA, 20 bp, Homo sapiens
  source 1..20: mol_type = genomic DNA
acagaaaggaagtggaagcc

SEQ ID NO: 3 - DNA, 20 bp, Homo sapiens
  source 1..20: mol_type = genomic DNA
cctacctttcaagacgaagt

SEQ ID NO: 4 - DNA, 20 bp, Homo sapiens
  source 1..20: mol_type = genomic DNA
cctttcaagacgaagtggca

SEQ ID NO: 5 - DNA, 20 bp, Homo sapiens
  source 1..20: mol_type = genomic DNA
aagacgaagtggcactacac

SEQ ID NO: 6 - DNA, 19 bp, Homo sapiens
  source 1..19: mol_type = genomic DNA
cgaagtggcactacaccag

SEQ ID NO: 7 - DNA, 20 bp, Homo sapiens
  source 1..20: mol_type = genomic DNA
acaccaggatgtgaaagtcc

SEQ ID NO: 8 - DNA, 20 bp, Homo sapiens
  source 1..20: mol_type = genomic DNA
caggatgtgaaagtccagcg

SEQ ID NO: 9 - DNA, 20 bp, Homo sapiens
  source 1..20: mol_type = genomic DNA
atgtgaaagtccagcgaaag

SEQ ID NO: 10 - DNA, 20 bp, Homo sapiens
  source 1..20: mol_type = genomic DNA
gaaagtccagcgaaagagac

SEQ ID NO: 11 - DNA, 20 bp, Homo sapiens
  source 1..20: mol_type = genomic DNA
gtccagcgaaagagacccaa

SEQ ID NO: 12 - DNA, 20 bp, Homo sapiens
  source 1..20: mol_type = genomic DNA
cccagaagccaagtctattc

SEQ ID NO: 13 - DNA, 20 bp, Homo sapiens
  source 1..20: mol_type = genomic DNA
cagaagccaagtctattcca

SEQ ID NO: 14 - DNA, 20 bp, Homo sapiens
  source 1..20: mol_type = genomic DNA
gaagccaagtctattccagg

SEQ ID NO: 15 - DNA, 20 bp, Homo sapiens
  source 1..20: mol_type = genomic DNA
gccaagtctattccaggcag

SEQ ID NO: 16 - DNA, 19 bp, Homo sapiens
  source 1..19: mol_type = genomic DNA
ggattagggtctgggctgg

SEQ ID NO: 17 - DNA, 20 bp, Homo sapiens
  source 1..20: mol_type = genomic DNA
cttgagtgaggtgggtgttg

SEQ ID NO: 18 - DNA, 20 bp, Homo sapiens
  source 1..20: mol_type = genomic DNA
gtgaggtgggtgttgctcta

SEQ ID NO: 19 - DNA, 20 bp, Homo sapiens
  source 1..20: mol_type = genomic DNA
ggtgggtgttgctctaattc

SEQ ID NO: 20 - DNA, 20 bp, Homo sapiens
  source 1..20: mol_type = genomic DNA
gttgctctaattcccctgtt

SEQ ID NO: 21 - DNA, 20 bp, synthetic construct
  source 1..20: mol_type = other DNA
catattgcgcgtatagtcgc

SEQ ID NO: 22 - DNA, 21 bp, synthetic construct
  source 1..21: mol_type = other DNA
ttccacttcctttctgtaagc

SEQ ID NO: 23 - DNA, 20 bp, synthetic construct
  source 1..20: mol_type = other DNA
ggcttccacttcctttctgt

SEQ ID NO: 24 - DNA, 20 bp, synthetic construct
  source 1..20: mol_type = other DNA
acttcgtcttgaaaggtagg

SEQ ID NO: 25 - DNA, 20 bp, synthetic construct
  source 1..20: mol_type = other DNA
tgccacttcgtcttgaaagg

SEQ ID NO: 26 - DNA, 20 bp, synthetic construct
  source 1..20: mol_type = other DNA
gtgtagtgccacttcgtctt

SEQ ID NO: 27 - DNA, 19 bp, synthetic construct
  source 1..19: mol_type = other DNA
ctggtgtagtgccacttcg

SEQ ID NO: 28 - DNA, 20 bp, synthetic construct
  source 1..20: mol_type = other DNA
ggactttcacatcctggtgt

SEQ ID NO: 29 - DNA, 20 bp, synthetic construct
  source 1..20: mol_type = other DNA
cgctggactttcacatcctg

SEQ ID NO: 30 - DNA, 20 bp, synthetic construct
  source 1..20: mol_type = other DNA
ctttcgctggactttcacat

SEQ ID NO: 31 - DNA, 20 bp, synthetic construct
  source 1..20: mol_type = other DNA
gtctctttcgctggactttc

SEQ ID NO: 32 - DNA, 20 bp, synthetic construct
  source 1..20: mol_type = other DNA
ttgggtctctttcgctggac

SEQ ID NO: 33 - DNA, 20 bp, synthetic construct
  source 1..20: mol_type = other DNA
gaatagacttggcttctggg

SEQ ID NO: 34 - DNA, 20 bp, synthetic construct
  source 1..20: mol_type = other DNA
tggaatagacttggcttctg

SEQ ID NO: 35 - DNA, 20 bp, synthetic construct
  source 1..20: mol_type = other DNA
cctggaatagacttggcttc

SEQ ID NO: 36 - DNA, 20 bp, synthetic construct
  source 1..20: mol_type = other DNA
ctgcctggaatagacttggc

SEQ ID NO: 37 - DNA, 19 bp, synthetic construct
  source 1..19: mol_type = other DNA
ccagcccagaccctaatcc

SEQ ID NO: 38 - DNA, 20 bp, synthetic construct
  source 1..20: mol_type = other DNA
caacacccacctcactcaag

SEQ ID NO: 39 - DNA, 20 bp, synthetic construct
  source 1..20: mol_type = other DNA
tagagcaacacccacctcac

SEQ ID NO: 40 - DNA, 20 bp, synthetic construct
  source 1..20: mol_type = other DNA
gaattagagcaacacccacc

SEQ ID NO: 41 - DNA, 20 bp, synthetic construct
  source 1..20: mol_type = other DNA
aacaggggaattagagcaac

SEQ ID NO: 42 - DNA, 20 bp, synthetic construct
  source 1..20: mol_type = other DNA
gcgactatacgcgcaatatg

SEQ ID NO: 43 - DNA, 20 bp, Homo sapiens
  source 1..20: mol_type = genomic DNA
cgagaaaccctacatctgca

SEQ ID NO: 44 - DNA, 20 bp, Homo sapiens
  source 1..20: mol_type = genomic DNA
tgagtcataaccagcctggc

SEQ ID NO: 45 - DNA, 20 bp, synthetic construct
  source 1..20: mol_type = other DNA
tgcagatgtagggtttctcg

SEQ ID NO: 46 - DNA, 20 bp, synthetic construct
  source 1..20: mol_type = other DNA
gccaggctggttatgactca

SEQ ID NO: 47 - DNA, 21 bp, Homo sapiens
  source 1..21: mol_type = genomic DNA
ttacagaaaggaagtggaagc

SEQ ID NO: 48 - DNA, 22 bp, Homo sapiens
  source 1..22: mol_type = genomic DNA
ttacagaaaggaagtggaagcc

SEQ ID NO: 49 - DNA, 20 bp, Homo sapiens
  source 1..20: mol_type = genomic DNA
tacagaaaggaagtggaagc

SEQ ID NO: 50 - DNA, 21 bp, Homo sapiens
  source 1..21: mol_type = genomic DNA
tacagaaaggaagtggaagcc

SEQ ID NO: 51 - DNA, 22 bp, Homo sapiens
  source 1..22: mol_type = genomic DNA
tacagaaaggaagtggaagccc

SEQ ID NO: 52 - DNA, 19 bp, Homo sapiens
  source 1..19: mol_type = genomic DNA
acagaaaggaagtggaagc

SEQ ID NO: 53 - DNA, 21 bp, Homo sapiens
  source 1..21: mol_type = genomic DNA
acagaaaggaagtggaagccc

SEQ ID NO: 54 - DNA, 18 bp, Homo sapiens
  source 1..18: mol_type = genomic DNA
cagaaaggaagtggaagc

SEQ ID NO: 55 - DNA, 19 bp, Homo sapiens
  source 1..19: mol_type = genomic DNA
cagaaaggaagtggaagcc

SEQ ID NO: 56 - DNA, 20 bp, Homo sapiens
  source 1..20: mol_type = genomic DNA
cagaaaggaagtggaagccc

SEQ ID NO: 57 - DNA, 17 bp, Homo sapiens
  source 1..17: mol_type = genomic DNA
agaaaggaagtggaagc

SEQ ID NO: 58 - DNA, 18 bp, Homo sapiens
  source 1..18: mol_type = genomic DNA
agaaaggaagtggaagcc

SEQ ID NO: 59 - DNA, 19 bp, Homo sapiens
  source 1..19: mol_type = genomic DNA
agaaaggaagtggaagccc

SEQ ID NO: 60 - DNA, 17 bp, Homo sapiens
  source 1..17: mol_type = genomic DNA
gaaaggaagtggaagcc

SEQ ID NO: 61 - DNA, 18 bp, Homo sapiens
  source 1..18: mol_type = genomic DNA
gaaaggaagtggaagccc

SEQ ID NO: 62 - DNA, 16 bp, Homo sapiens
  source 1..16: mol_type = genomic DNA
aaaggaagtggaagcc

SEQ ID NO: 63 - DNA, 17 bp, Homo sapiens
  source 1..17: mol_type = genomic DNA
aaaggaagtggaagccc

SEQ ID NO: 64 - DNA, 16 bp, Homo sapiens
  source 1..16: mol_type = genomic DNA
aaggaagtggaagccc

SEQ ID NO: 65 - DNA, 20 bp, Homo sapiens
  source 1..20: mol_type = genomic DNA
gtggcactacaccaggatgt

SEQ ID NO: 66 - DNA, 20 bp, Homo sapiens
  source 1..20: mol_type = genomic DNA
ggcactacaccaggatgtga

SEQ ID NO: 67 - DNA, 20 bp, Homo sapiens
  source 1..20: mol_type = genomic DNA
cactacaccaggatgtgaaa

SEQ ID NO: 68 - DNA, 20 bp, Homo sapiens
  source 1..20: mol_type = genomic DNA
ctacaccaggatgtgaaagt

SEQ ID NO: 69 - DNA, 21 bp, synthetic construct
  source 1..21: mol_type = other DNA
gcttccacttcctttctgtaa

SEQ ID NO: 70 - DNA, 22 bp, synthetic construct
  source 1..22: mol_type = other DNA
ggcttccacttcctttctgtaa

SEQ ID NO: 71 - DNA, 20 bp, synthetic construct
  source 1..20: mol_type = other DNA
gcttccacttcctttctgta

SEQ ID NO: 72 - DNA, 21 bp, synthetic construct
  source 1..21: mol_type = other DNA
ggcttccacttcctttctgta

SEQ ID NO: 73 - DNA, 22 bp, synthetic construct
  source 1..22: mol_type = other DNA
gggcttccacttcctttctgta

SEQ ID NO: 74 - DNA, 19 bp, synthetic construct
  source 1..19: mol_type = other DNA
gcttccacttcctttctgt

SEQ ID NO: 75 - DNA, 21 bp, synthetic construct
  source 1..21: mol_type = other DNA
gggcttccacttcctttctgt

SEQ ID NO: 76 - DNA, 18 bp, synthetic construct
  source 1..18: mol_type = other DNA
gcttccacttcctttctg

SEQ ID NO: 77 - DNA, 19 bp, synthetic construct
  source 1..19: mol_type = other DNA
ggcttccacttcctttctg

SEQ ID NO: 78 - DNA, 20 bp, synthetic construct
  source 1..20: mol_type = other DNA
gggcttccacttcctttctg

SEQ ID NO: 79 - DNA, 17 bp, synthetic construct
  source 1..17: mol_type = other DNA
gcttccacttcctttct

SEQ ID NO: 80 - DNA, 18 bp, synthetic construct
  source 1..18: mol_type = other DNA
ggcttccacttcctttct

SEQ ID NO: 81 - DNA, 19 bp, synthetic construct
  source 1..19: mol_type = other DNA
gggcttccacttcctttct

SEQ ID NO: 82 - DNA, 17 bp, synthetic construct
  source 1..17: mol_type = other DNA
ggcttccacttcctttc

SEQ ID NO: 83 - DNA, 18 bp, synthetic construct
  source 1..18: mol_type = other DNA
gggcttccacttcctttc

SEQ ID NO: 84 - DNA, 16 bp, synthetic construct
  source 1..16: mol_type = other DNA
ggcttccacttccttt

SEQ ID NO: 85 - DNA, 17 bp, synthetic construct
  source 1..17: mol_type = other DNA
gggcttccacttccttt

SEQ ID NO: 86 - DNA, 16 bp, synthetic construct
  source 1..16: mol_type = other DNA
gggcttccacttcctt

SEQ ID NO: 87 - DNA, 20 bp, synthetic construct
  source 1..20: mol_type = other DNA
acatcctggtgtagtgccac

SEQ ID NO: 88 - DNA, 20 bp, synthetic construct
  source 1..20: mol_type = other DNA
tcacatcctggtgtagtgcc

SEQ ID NO: 89 - DNA, 20 bp, synthetic construct
  source 1..20: mol_type = other DNA
tttcacatcctggtgtagtg

SEQ ID NO: 90 - DNA, 20 bp, synthetic construct
  source 1..20: mol_type = other DNA
actttcacatcctggtgtag

SEQ ID NO: 91 - DNA, 21 bp, Homo sapiens
  source 1..21: mol_type = genomic DNA
ttttacctgtactttcttcag

SEQ ID NO: 92 - DNA, 20 bp, Homo sapiens
  source 1..20: mol_type = genomic DNA
cctgtactttcttcagggta

SEQ ID NO: 93 - DNA, 21 bp, Homo sapiens
  source 1..21: mol_type = genomic DNA
gtactttcttcagggtatcct

SEQ ID NO: 94 - DNA, 20 bp, Homo sapiens
  source 1..20: mol_type = genomic DNA
ttcttcagggtatcctgtct

SEQ ID NO: 95 - DNA, 20 bp, Homo sapiens
  source 1..20: mol_type = genomic DNA
tcttggtagtgaatggaaga

SEQ ID NO: 96 - DNA, 20 bp, Homo sapiens
  source 1..20: mol_type = genomic DNA
ggcagtgcagaaggcacttt

SEQ ID NO: 97 - DNA, 20 bp, Homo sapiens
  source 1..20: mol_type = genomic DNA
gcagaaggcactttgatcat

SEQ ID NO: 98 - DNA, 22 bp, Homo sapiens
  source 1..22: mol_type = genomic DNA
taagagatccaattaagaagaa

SEQ ID NO: 99 - DNA, 22 bp, Homo sapiens
  source 1..22: mol_type = genomic DNA
gagatccaattaagaagaatag

SEQ ID NO: 100 - DNA, 19 bp, Homo sapiens
  source 1..19: mol_type = genomic DNA
accagcccagagtggcttc

SEQ ID NO: 101 - DNA, 19 bp, Homo sapiens
  source 1..19: mol_type = genomic DNA
cgctcagctggtacgtttg

SEQ ID NO: 102 - DNA, 20 bp, Homo sapiens
  source 1..20: mol_type = genomic DNA
gctggtacgtttgtgtttgt

SEQ ID NO: 103 - DNA, 21 bp, Homo sapiens
  source 1..21: mol_type = genomic DNA
tggtacgtttgtgtttgtcat

SEQ ID NO: 104 - DNA, 21 bp, Homo sapiens
  source 1..21: mol_type = genomic DNA
acgtttgtgtttgtcattagg

SEQ ID NO: 105 - DNA, 22 bp, Homo sapiens
  source 1..22: mol_type = genomic DNA
gccctcaacaagcactaacatt

SEQ ID NO: 106 - DNA, 21 bp, synthetic construct
  source 1..21: mol_type = other DNA
ctgaagaaagtacaggtaaaa

SEQ ID NO: 107 - DNA, 20 bp, synthetic construct
  source 1..20: mol_type = other DNA
taccctgaagaaagtacagg

SEQ ID NO: 108 - DNA, 21 bp, synthetic construct
  source 1..21: mol_type = other DNA
aggataccctgaagaaagtac

SEQ ID NO: 109 - DNA, 20 bp, synthetic construct
  source 1..20: mol_type = other DNA
agacaggataccctgaagaa

SEQ ID NO: 110 - DNA, 20 bp, synthetic construct
  source 1..20: mol_type = other DNA
tcttccattcactaccaaga

SEQ ID NO: 111 - DNA, 20 bp, synthetic construct
  source 1..20: mol_type = other DNA
aaagtgccttctgcactgcc

SEQ ID NO: 112 - DNA, 20 bp, synthetic construct
  source 1..20: mol_type = other DNA
atgatcaaagtgccttctgc

SEQ ID NO: 113 - DNA, 22 bp, synthetic construct
  source 1..22: mol_type = other DNA
ttcttcttaattggatctctta

SEQ ID NO: 114 - DNA, 22 bp, synthetic construct
  source 1..22: mol_type = other DNA
ctattcttcttaattggatctc

SEQ ID NO: 115 - DNA, 19 bp, synthetic construct
  source 1..19: mol_type = other DNA
gaagccactctgggctggt

SEQ ID NO: 116 - DNA, 19 bp, synthetic construct
  source 1..19: mol_type = other DNA
caaacgtaccagctgagcg

SEQ ID NO: 117 - DNA, 20 bp, synthetic construct
  source 1..20: mol_type = other DNA
acaaacacaaacgtaccagc

SEQ ID NO: 118 - DNA, 21 bp, synthetic construct
  source 1..21: mol_type = other DNA
atgacaaacacaaacgtacca

SEQ ID NO: 119 - DNA, 21 bp, synthetic construct
  source 1..21: mol_type = other DNA
cctaatgacaaacacaaacgt

SEQ ID NO: 120 - DNA, 22 bp, synthetic construct
  source 1..22: mol_type = other DNA
aatgttagtgcttgttgagggc

SEQ ID NO: 121 - DNA, 21 bp, Homo sapiens
  source 1..21: mol_type = genomic DNA
tgcagaaggcactttgatcat

SEQ ID NO: 122 - DNA, 21 bp, Homo sapiens
  source 1..21: mol_type = genomic DNA
cagaaggcactttgatcatct

SEQ ID NO: 123 - DNA, 21 bp, Homo sapiens
  source 1..21: mol_type = genomic DNA
gaaggcactttgatcatctca

SEQ ID NO: 124 - DNA, 20 bp, Homo sapiens
  source 1..20: mol_type = genomic DNA
ggcactttgatcatctcact

SEQ ID NO: 125 - DNA, 20 bp, Homo sapiens
  source 1..20: mol_type = genomic DNA
ctttgatcatctcactcact

SEQ ID NO: 126 - DNA, 21 bp, Homo sapiens
  source 1..21: mol_type = genomic DNA
atcatctcactcactgcaaat

SEQ ID NO: 127 - DNA, 20 bp, Homo sapiens
  source 1..20: mol_type = genomic DNA
atctcactcactgcaaatgt

SEQ ID NO: 128 - DNA, 22 bp, Homo sapiens
  source 1..22: mol_type = genomic DNA
attaagagatccaattaagaag

SEQ ID NO: 129 - DNA, 22 bp, Homo sapiens
  source 1..22: mol_type = genomic DNA
ttaagagatccaattaagaaga

SEQ ID NO: 130 - DNA, 20 bp, Homo sapiens
  source 1..20: mol_type = genomic DNA
cagtgcagaaggcactttga

SEQ ID NO: 131 - DNA, 22 bp, Homo sapiens
  source 1..22: mol_type = genomic DNA
tgcagaaggcactttgatcatc

SEQ ID NO: 132 - DNA, 19 bp, Homo sapiens
  source 1..19: mol_type = genomic DNA
cagaaggcactttgatcat

SEQ ID NO: 133 - DNA, 18 bp, Homo sapiens
  source 1..18: mol_type = genomic DNA
agaaggcactttgatcat

SEQ ID NO: 134 - DNA, 25 bp, Homo sapiens
  source 1..25: mol_type = genomic DNA
actttgatcatctcactcactgcaa

SEQ ID NO: 135 - DNA, 20 bp, Homo sapiens
  source 1..20: mol_type = genomic DNA
ttgatcatctcactcactgc

SEQ ID NO: 136 - DNA, 20 bp, Homo sapiens
  source 1..20: mol_type = genomic DNA
tgatcatctcactcactgca

SEQ ID NO: 137 - DNA, 18 bp, Homo sapiens
  source 1..18: mol_type = genomic DNA
atcatctcactcactgca

SEQ ID NO: 138 - DNA, 20 bp, Homo sapiens
  source 1..20: mol_type = genomic DNA
catctcactcactgcaaatg

SEQ ID NO: 139 - DNA, 22 bp, Homo sapiens
  source 1..22: mol_type = genomic DNA
gtattaagagatccaattaaga

SEQ ID NO: 140 - DNA, 25 bp, Homo sapiens
  source 1..25: mol_type = genomic DNA
gtattaagagatccaattaagaaga

SEQ ID NO: 141 - DNA, 18 bp, Homo sapiens
  source 1..18: mol_type = genomic DNA
cgagcgtgattaaactaa

SEQ ID NO: 142 - DNA, 21 bp, synthetic construct
  source 1..21: mol_type = other DNA
atgatcaaagtgccttctgca

SEQ ID NO: 143 - DNA, 21 bp, synthetic construct
  source 1..21: mol_type = other DNA
agatgatcaaagtgccttctg

SEQ ID NO: 144 - DNA, 21 bp, synthetic construct
  source 1..21: mol_type = other DNA
tgagatgatcaaagtgccttc

SEQ ID NO: 145 - DNA, 20 bp, synthetic construct
  source 1..20: mol_type = other DNA
agtgagatgatcaaagtgcc

SEQ ID NO: 146 - DNA, 20 bp, synthetic construct
  source 1..20: mol_type = other DNA
agtgagtgagatgatcaaag

SEQ ID NO: 147 - DNA, 21 bp, synthetic construct
  source 1..21: mol_type = other DNA
atttgcagtgagtgagatgat

SEQ ID NO: 148 - DNA, 20 bp, synthetic construct
  source 1..20: mol_type = other DNA
acatttgcagtgagtgagat

SEQ ID NO: 149 - DNA, 22 bp, synthetic construct
  source 1..22: mol_type = other DNA
cttcttaattggatctcttaat

SEQ ID NO: 150 - DNA, 22 bp, synthetic construct
  source 1..22: mol_type = other DNA
tcttcttaattggatctcttaa

SEQ ID NO: 151 - DNA, 20 bp, synthetic construct
  source 1..20: mol_type = other DNA
tcaaagtgccttctgcactg

SEQ ID NO: 152 - DNA, 22 bp, synthetic construct
  source 1..22: mol_type = other DNA
gatgatcaaagtgccttctgca

SEQ ID NO: 153 - DNA, 19 bp, synthetic construct
  source 1..19: mol_type = other DNA
atgatcaaagtgccttctg

SEQ ID NO: 154 - DNA, 18 bp, synthetic construct
  source 1..18: mol_type = other DNA
atgatcaaagtgccttct

SEQ ID NO: 155 - DNA, 25 bp, synthetic construct
  source 1..25: mol_type = other DNA
ttgcagtgagtgagatgatcaaagt

SEQ ID NO: 156 - DNA, 20 bp, synthetic construct
  source 1..20: mol_type = other DNA
gcagtgagtgagatgatcaa

SEQ ID NO: 157 - DNA, 20 bp, synthetic construct
  source 1..20: mol_type = other DNA
tgcagtgagtgagatgatca

SEQ ID NO: 158 - DNA, 18 bp, synthetic construct
  source 1..18: mol_type = other DNA
tgcagtgagtgagatgat

SEQ ID NO: 159 - DNA, 20 bp, synthetic construct
  source 1..20: mol_type = other DNA
catttgcagtgagtgagatg

SEQ ID NO: 160 - DNA, 22 bp, synthetic construct
  source 1..22: mol_type = other DNA
tcttaattggatctcttaatac

SEQ ID NO: 161 - DNA, 25 bp, synthetic construct
  source 1..25: mol_type = other DNA
tcttcttaattggatctcttaatac

SEQ ID NO: 162 - DNA, 18 bp, synthetic construct
  source 1..18: mol_type = other DNA
ttagtttaatcacgctcg

SEQ ID NO: 163 - DNA, 20 bp, synthetic construct
  source 1..20: mol_type = other DNA
acatgttggatgaggctctg

SEQ ID NO: 164 - DNA, 24 bp, synthetic construct
  source 1..24: mol_type = other DNA
ctcttctcattaactgctggacta

SEQ ID NO: 165 - DNA, 20 bp, synthetic construct
  source 1..20: mol_type = other DNA
ctggatcagaccctgaatct

SEQ ID NO: 166 - DNA, 20 bp, synthetic construct
  source 1..20: mol_type = other DNA
cctctgagtggtcccataat

SEQ ID NO: 167 - DNA, 21 bp, synthetic construct
  source 1..21: mol_type = other DNA
tggaggctagtccagcagtta

SEQ ID NO: 168 - DNA, 23 bp, synthetic construct
  source 1..23: mol_type = other DNA
ggtgtgaaccatgagaagtatga

SEQ ID NO: 169 - DNA, 22 bp, synthetic construct
  source 1..22: mol_type = other DNA
gagtccttccacgataccaaag

SEQ ID NO: 170 - DNA, 24 bp, synthetic construct
  source 1..24: mol_type = other DNA
agatcatcagcaatgcctcctgca

SEQ ID NO: 171 - DNA, 20 bp, synthetic construct
  source 1..20: mol_type = other DNA
aattggaccccgtgattccc

SEQ ID NO: 172 - DNA, 17 bp, synthetic construct
  source 1..17: mol_type = other DNA
gtcctcgacacccatgc

SEQ ID NO: 173 - DNA, 225 bp, Homo sapiens
  source 1..225: mol_type = genomic DNA
aaaggaagtggaagccccctacctttcaagacgaagtggcactacaccaggatgtgaaagtccagcgaaagagacccaaggggcctagggggcagcacacccccagaagccaagtctattccaggcagtaccagggattagggtctgggctggaaaaatcctggtgttttgaatatgttcaggtccagttcagactcttgatcccacagccacttcttgagtgag

SEQ ID NO: 174 - DNA, 193 bp, Homo sapiens
  source 1..193: mol_type = genomic DNA
ggtatcctgtcttggtagtgaatggaagagggcctggtccctggggcagtgcagaaggcactttgatcatctcactcactgcaaatgtcatgtgaggtttcatggaagtattaagagatccaattaagaagaatagttctgagtctaaaccagcccagagtggcttctctaggggaaactccccgctcagctg